European Patent Application EP 4 234 574 A1, published August 30, 2023. Title: CRF2 RECEPTOR AGONISTS AND THEIR USE IN THERAPY. Applicant: Corteria Pharmaceuticals. The sequence listing filed with the application follows.

SEQUENCE LISTING (151 sequences)

SEQ ID NO: 1 - protein, 38 aa, synthetic construct
  VARIANT 1: absent or I
  VARIANT 2: Valine or D-valine
  VARIANT 7: Valine or D-valine
  VARIANT 11: L or I or alpha-methyl-leucien or Aib
  MOD_RES 12: the epsilon-amino group of the lysine side chain is covalently bound to an albumin -binding moiety
  VARIANT 13: K or Q
  VARIANT 14: I or Aib
  VARIANT 15: L or alpha-methyl-leucine or Aib
  VARIANT 17: E or K
  VARIANT 20: K or R
  VARIANT 23: K or A or Aib
  VARIANT 25: R or alpha-methyl-leucine or Aib
  VARIANT 26: E or Aib
  VARIANT 30: K or T
  VARIANT 31: N or Q or A
  VARIANT 32: K or V or T or Aib or E or A or Abu or Nva or alpha-methyl-leucine or Dap or 4-Pip or Thp or Chx or Cpex or Cpx
  VARIANT 36: A or E
XXLSLDXPIKXKXXXLXQEXQKXQXXQAEXXXQILXQV

SEQ ID NO: 2 - protein, 38 aa, synthetic construct
  MOD_RES 1: ACETYLATION
  VARIANT 7: D-valine
  MOD_RES 12: the epsilon-amino group of the lysine side chain is covalently bound to an albumin -binding moiety
  MOD_RES 38: AMIDATION
IVLSLDXPIKLKQILLKQERQKKQREQAEKNKQILEQV

SEQ ID NO: 3 - protein, 37 aa, synthetic construct
  MOD_RES 1: ACETYLATION
  VARIANT 6: D-valine
  MOD_RES 11: the epsilon-amino group of the lysine side chain is covalently bound to an albumin -binding moiety
  MOD_RES 37: AMIDATION
VLSLDXPIKLKQILLKQERQKKQREQAEKNKQILEQV

SEQ ID NO: 4 - protein, 37 aa, synthetic construct; identical to SEQ ID NO: 3
  VARIANT 6: D-valine
  MOD_RES 11: the epsilon-amino group of the lysine side chain is covalently bound to an albumin -binding moiety
  MOD_RES 37: AMIDATION

SEQ ID NO: 5 - protein, 38 aa, synthetic construct; identical to SEQ ID NO: 2
  MOD_RES 1: met
  VARIANT 7: D-valine
  MOD_RES 12: the epsilon-amino group of the lysine side chain is covalently bound to an albumin -binding moiety
  MOD_RES 38: AMIDATION

SEQ ID NO: 6 - protein, 37 aa, synthetic construct
  MOD_RES 1: Acetylated with a propanoyl group
  VARIANT 6: D-valine
  MOD_RES 11: the epsilon-amino group of the lysine side chain is covalently bound to an albumin -binding moiety
  MOD_RES 37: AMIDATION
VLSLDVPIKLKQILLKQERQKKQREQAEKNKQILEQV

SEQ ID NO: 7 - protein, 37 aa, synthetic construct; identical to SEQ ID NO: 6
  MOD_RES 1: Acetylated with a butanoyl group
  VARIANT 6: D-valine
  MOD_RES 11: the epsilon-amino group of the lysine side chain is covalently bound to an albumin -binding moiety
  MOD_RES 37: AMIDATION

SEQ ID NO: 8 - protein, 37 aa, synthetic construct; identical to SEQ ID NO: 6
  MOD_RES 1: Acetylated with a pentanoyl group
  VARIANT 6: D-valine
  MOD_RES 11: the epsilon-amino group of the lysine side chain is covalently bound to an albumin -binding moiety
  MOD_RES 37: AMIDATION

SEQ ID NO: 9 - protein, 37 aa, synthetic construct; identical to SEQ ID NO: 6
  MOD_RES 1: Acetylated with a isopentanoyl group
  VARIANT 6: D-valine
  MOD_RES 11: the epsilon-amino group of the lysine side chain is covalently bound to an albumin -binding moiety
  MOD_RES 37: AMIDATION

SEQ ID NO: 10 - protein, 38 aa, synthetic construct
  VARIANT 7: D-valine
  MOD_RES 12: the epsilon-amino group of the lysine side chain is covalently bound to an albumin -binding moiety
  VARIANT 32: X is Aib
  MOD_RES 38: AMIDATION
IVLSLDVPIKLKQILLKQERQKKQREQAEKNXQILEQV

SEQ ID NO: 11 - protein, 38 aa, synthetic construct
  VARIANT 7: D-valine
  MOD_RES 12: the epsilon-amino group of the lysine side chain is covalently bound to an albumin -binding moiety
  VARIANT 32: X is Aib
  MOD_RES 38: AMIDATION
IVLSLDVPIKLKKILLEQEKQKKQREQAETNXQILAQV

SEQ ID NO: 12 - protein, 38 aa, synthetic construct; identical to SEQ ID NO: 11
  VARIANT 7: D-valine
  MOD_RES 12: the epsilon-amino group of the lysine side chain is covalently bound to an albumin -binding moiety
  VARIANT 32: X is Aib
  MOD_RES 38: AMIDATION

SEQ ID NO: 13 - protein, 38 aa, synthetic construct
  VARIANT 7: D-valine
  MOD_RES 12: the epsilon-amino group of the lysine side chain is covalently bound to an albumin -binding moiety
  MOD_RES 38: AMIDATION
IVLSLDVPIKLKQILLKQERQKKQREQAEKNVQILEQV

SEQ ID NO: 14 - protein, 38 aa, synthetic construct
  VARIANT 7: D-valine
  MOD_RES 12: the epsilon-amino group of the lysine side chain is covalently bound to an albumin -binding moiety
  MOD_RES 38: AMIDATION
IVLSLDVPIKLKQILLKQERQKKQREQAEKNTQILEQV

SEQ ID NO: 15 - protein, 37 aa, synthetic construct
  VARIANT 6: D-valine
  MOD_RES 11: the epsilon-amino group of the lysine side chain is covalently bound to an albumin -binding moiety
  VARIANT 22: X is Aib
  VARIANT 31: X is Aib
  MOD_RES 37: AMIDATION
VLSLDVPIKLKKILLEQEKQKXQREQAETNXQILAQV

SEQ ID NO: 16 - protein, 38 aa, synthetic construct; identical to SEQ ID NO: 10
  MOD_RES 1: ACETYLATION
  VARIANT 7: D-valine
  MOD_RES 12: the epsilon-amino group of the lysine side chain is covalently bound to an albumin -binding moiety
  VARIANT 32: X is Aib
  MOD_RES 38: AMIDATION

SEQ ID NO: 17 - protein, 38 aa, synthetic construct
  MOD_RES 1: ACETYLATION
  VARIANT 7: D-valine
  MOD_RES 12: the epsilon-amino group of the lysine side chain is covalently bound to an albumin -binding moiety
  MOD_RES 38: AMIDATION
IVLSLDVPIKLKQILLKQERQKKQREQAEKNEQILEQV

SEQ ID NO: 18 - protein, 38 aa, synthetic construct
  MOD_RES 1: ACETYLATION
  VARIANT 7: D-valine
  MOD_RES 12: the epsilon-amino group of the lysine side chain is covalently bound to an albumin -binding moiety
  VARIANT 14: X is Aib
  MOD_RES 38: AMIDATION
IVLSLDVPIKLKQXLLKQERQKKQREQAEKNVQILEQV

SEQ ID NO: 19 - protein, 38 aa, synthetic construct
  MOD_RES 1: ACETYLATION
  VARIANT 11: X is alpha-methyl-leucine
  MOD_RES 12: the epsilon-amino group of the lysine side chain is covalently bound to an albumin -binding moiety
  VARIANT 32: X is Aib
  MOD_RES 38: AMIDATION
IVLSLDVPIKXKQILLKQERQKKQREQAEKNXQILEQV

SEQ ID NO: 20 - protein, 38 aa, synthetic construct
  MOD_RES 1: ACETYLATION
  VARIANT 11: X is alpha-methyl-leucine
  MOD_RES 12: the epsilon-amino group of the lysine side chain is covalently bound to an albumin -binding moiety
  VARIANT 14: X is Aib
  MOD_RES 38: AMIDATION
IVLSLDVPIKXKQXLLKQERQKKQREQAEKNXQILEQV

SEQ ID NO: 21 - protein, 38 aa, synthetic construct
  MOD_RES 1: ACETYLATION
  VARIANT 7: D-valine
  MOD_RES 12: the epsilon-amino group of the lysine side chain is covalently bound to an albumin -binding moiety
  VARIANT 32: X is Aib
  MOD_RES 38: AMIDATION
IVLSLDVPIKLKKILLKQERQKKQREQAEKNXQILEQV

SEQ ID NO: 22 - protein, 37 aa, synthetic construct
  MOD_RES 1: Acetylated with a pentanoyl group
  VARIANT 6: D-valine
  MOD_RES 11: the epsilon-amino group of the lysine side chain is covalently bound to an albumin -binding moiety
  VARIANT 14: X is Aib
  MOD_RES 37: AMIDATION
VLSLDVPIKLKQXLLKQERQKKQREQAEKNVQILEQV

SEQ ID NO: 23 - protein, 38 aa, synthetic construct; identical to SEQ ID NO: 10
  MOD_RES 1: METHYLATION
  VARIANT 7: D-valine
  MOD_RES 12: the epsilon-amino group of the lysine side chain is covalently bound to an albumin -binding moiety
  VARIANT 32: X is Aib
  MOD_RES 38: AMIDATION

SEQ ID NO: 24 - protein, 38 aa, synthetic construct
  MOD_RES 1: METHYLATION
  VARIANT 7: D-valine
  MOD_RES 12: the epsilon-amino group of the lysine side chain is covalently bound to an albumin -binding moiety
  MOD_RES 38: AMIDATION
IVLSLDVPIKLKQILLKQERQKKQREQAEKNAQILEQV

SEQ ID NO: 25 - protein, 38 aa, synthetic construct
  MOD_RES 12: the epsilon-amino group of the lysine side chain is covalently bound to an albumin -binding moiety
  VARIANT 14: X is Aib
  VARIANT 32: X is Aib
  MOD_RES 38: AMIDATION
IVLSLDVPIKLKQXLLKQERQKKQREQAEKNXQILEQV

SEQ ID NO: 26 - protein, 38 aa, synthetic construct; identical to SEQ ID NO: 25
  MOD_RES 1: ACETYLATION
  MOD_RES 12: the epsilon-amino group of the lysine side chain is covalently bound to an albumin -binding moiety
  VARIANT 14: X is Aib
  VARIANT 32: X is Aib
  MOD_RES 38: AMIDATION

SEQ ID NO: 27 - protein, 38 aa, synthetic construct; identical to SEQ ID NO: 18
  MOD_RES 1: ACETYLATION
  VARIANT 7: D-valine
  MOD_RES 12: the epsilon-amino group of the lysine side chain is covalently bound to an albumin -binding moiety
  VARIANT 14: X is Aib
  MOD_RES 38: AMIDATION

SEQ ID NO: 28 - protein, 38 aa, synthetic construct; identical to SEQ ID NO: 18
  MOD_RES 1: METHYLATION
  VARIANT 7: D-valine
  MOD_RES 12: the epsilon-amino group of the lysine side chain is covalently bound to an albumin -binding moiety
  VARIANT 14: X is Aib
  MOD_RES 38: AMIDATION

SEQ ID NO: 29 - protein, 37 aa, synthetic construct; identical to SEQ ID NO: 22
  MOD_RES 1: Acetylated with a pentanoyl group
  VARIANT 6: D-valine
  MOD_RES 11: the epsilon-amino group of the lysine side chain is covalently bound to an albumin -binding moiety
  VARIANT 13: X is Aib
  MOD_RES 37: AMIDATION

SEQ ID NO: 30 - protein, 38 aa, synthetic construct; identical to SEQ ID NO: 10
  MOD_RES 1: ACETYLATION
  VARIANT 7: D-valine
  MOD_RES 12: the epsilon-amino group of the lysine side chain is covalently bound to an albumin -binding moiety
  VARIANT 32: X is Aib
  MOD_RES 38: AMIDATION

SEQ ID NO: 31 - protein, 38 aa, synthetic construct; identical to SEQ ID NO: 10
  MOD_RES 1: METHYLATION
  VARIANT 7: D-valine
  MOD_RES 12: the epsilon-amino group of the lysine side chain is covalently bound to an albumin -binding moiety
  VARIANT 32: X is Aib
  MOD_RES 38: AMIDATION

SEQ ID NO: 32 - protein, 37 aa, synthetic construct
  MOD_RES 1: Acetylated with a pentanoyl group
  VARIANT 6: D-valine
  MOD_RES 11: the epsilon-amino group of the lysine side chain is covalently bound to an albumin -binding moiety
  VARIANT 31: X is Aib
  MOD_RES 37: AMIDATION
VLSLDVPIKLKQILLKQERQKKQREQAEKNXQILEQV

SEQ ID NO: 33 - protein, 37 aa, synthetic construct
  MOD_RES 1: ACETYLATION
  VARIANT 6: D-valine
  MOD_RES 11: the epsilon-amino group of the lysine side chain is covalently bound to an albumin -binding moiety
  MOD_RES 37: AMIDATION
VLSLDVPIKLKKILLEQEKQKKQREQAETNKQILAQV

SEQ ID NO: 34 - protein, 37 aa, synthetic construct; identical to SEQ ID NO: 33
  VARIANT 6: D-valine
  VARIANT 11: the epsilon-amino group of the lysine side chain is covalently bound to an albumin -binding moiety
  MOD_RES 37: AMIDATION

SEQ ID NO: 35 - protein, 37 aa, synthetic construct; identical to SEQ ID NO: 33
  MOD_RES 1: Acetylated with a propanoyl group
  VARIANT 6: D-valine
  MOD_RES 11: the epsilon-amino group of the lysine side chain is covalently bound to an albumin -binding moiety
  MOD_RES 37: AMIDATION

SEQ ID NO: 36 - protein, 37 aa, synthetic construct; identical to SEQ ID NO: 33
  MOD_RES 1: Acetylated with a butanoyl group
  VARIANT 6: D-valine
  MOD_RES 11: the epsilon-amino group of the lysine side chain is covalently bound to an albumin -binding moiety
  MOD_RES 37: AMIDATION

SEQ ID NO: 37 - protein, 37 aa, synthetic construct; identical to SEQ ID NO: 33
  MOD_RES 1: Acetylated with a pentanoyl group
  VARIANT 6: D-valine
  MOD_RES 11: the epsilon-amino group of the lysine side chain is covalently bound to an albumin -binding moiety
  MOD_RES 37: AMIDATION

SEQ ID NO: 38 - protein, 38 aa, synthetic construct
  VARIANT 11: X is alpha-methyl-leucine
  MOD_RES 12: the epsilon-amino group of the lysine side chain is covalently bound to an albumin -binding moiety
  VARIANT 32: X is Aib
  MOD_RES 38: AMIDATION
IVLSLDVPIKXKKILLEQEKQKKQREQAETNXQILAQV

SEQ ID NO: 39 - protein, 38 aa, synthetic construct; identical to SEQ ID NO: 11
  MOD_RES 1: ACETYLATION
  MOD_RES 12: the epsilon-amino group of the lysine side chain is covalently bound to an albumin -binding moiety
  VARIANT 32: X is Aib
  MOD_RES 38: AMIDATION

SEQ ID NO: 40 - protein, 38 aa, synthetic construct; identical to SEQ ID NO: 11
  MOD_RES 1: ACETYLATION
  VARIANT 7: D-valine
  MOD_RES 12: the epsilon-amino group of the lysine side chain is covalently bound to an albumin -binding moiety
  VARIANT 32: X is Aib
  MOD_RES 38: AMIDATION

SEQ ID NO: 41 - protein, 38 aa, synthetic construct; identical to SEQ ID NO: 11
  MOD_RES 1: ACETYLATION
  VARIANT 7: D-valine
  MOD_RES 12: the epsilon-amino group of the lysine side chain is covalently bound to an albumin -binding moiety
  VARIANT 32: x is Aib
  MOD_RES 38: AMIDATION

SEQ ID NO: 42 - protein, 38 aa, synthetic construct; identical to SEQ ID NO: 11
  MOD_RES 1: ACETYLATION
  VARIANT 7: D-valine
  MOD_RES 12: the epsilon-amino group of the lysine side chain is covalently bound to an albumin -binding moiety
  VARIANT 32: X is Aib
  MOD_RES 38: AMIDATION

SEQ ID NO: 43 - protein, 38 aa, synthetic construct; identical to SEQ ID NO: 38
  MOD_RES 1: ACETYLATION
  VARIANT 11: X is alpha-methyl-leucine
  MOD_RES 12: the epsilon-amino group of the lysine side chain is covalently bound to an albumin -binding moiety
  VARIANT 32: X is Aib
  MOD_RES 38: AMIDATION

SEQ ID NO: 44 - protein, 38 aa, synthetic construct; identical to SEQ ID NO: 38
  MOD_RES 1: ACETYLATION
  VARIANT 7: D-valine
  VARIANT 11: X is alpha-methyl-leucine
  MOD_RES 12: the epsilon-amino group of the lysine side chain is covalently bound to an albumin -binding moiety
  VARIANT 32: X is Aib
  MOD_RES 38: AMIDATION

SEQ ID NO: 45 - protein, 37 aa, synthetic construct
  MOD_RES 1: ACETYLATION
  VARIANT 6: D-valine
  MOD_RES 11: the epsilon-amino group of the lysine side chain is covalently bound to an albumin -binding moiety
  VARIANT 31: X is Aib
  MOD_RES 37: AMIDATION
VLSLDVPIKLKKILLEQEKQKKQREQAETNXQILAQV

SEQ ID NO: 46 - protein, 37 aa, synthetic construct
  MOD_RES 1: ACETYLATION
  VARIANT 6: D-valine
  VARIANT 10: X is alpha-methyl-leucine
  MOD_RES 11: the epsilon-amino group of the lysine side chain is covalently bound to an albumin -binding moiety
  VARIANT 31: X is Aib
  MOD_RES 37: AMIDATION
VLSLDVPIKXKKILLEQEKQKKQREQAETNXQILAQV

SEQ ID NO: 47 - protein, 38 aa, synthetic construct
  MOD_RES 1: ACETYLATION
  VARIANT 7: D-valine
  MOD_RES 12: the epsilon-amino group of the lysine side chain is covalently bound to an albumin -binding moiety
  MOD_RES 38: AMIDATION
IVLSLDVPIKLKKILLEQEKQKKQREQAETNAQILAQV

SEQ ID NO: 48 - protein, 38 aa, synthetic construct
  MOD_RES 1: ACETYLATION
  VARIANT 7: D-valine
  MOD_RES 12: the epsilon-amino group of the lysine side chain is covalently bound to an albumin -binding moiety
  MOD_RES 38: AMIDATION
IVLSLDVPIKLKKILLEQEKQKKQREQAETNVQILAQV

SEQ ID NO: 49 - protein, 38 aa, synthetic construct
  MOD_RES 1: ACETYLATION
  VARIANT 11: X is alpha-methyl-leucine
  MOD_RES 12: the epsilon-amino group of the lysine side chain is covalently bound to an albumin -binding moiety
  MOD_RES 38: ACETYLATION
IVLSLDVPIKXKKILLEQEKQKKQREQAETNVQILAQV

SEQ ID NO: 50 - protein, 38 aa, synthetic construct; identical to SEQ ID NO: 49
  MOD_RES 1: ACETYLATION
  VARIANT 7: D-valine
  VARIANT 11: X is alpha-methyl-leucine
  MOD_RES 12: the epsilon-amino group of the lysine side chain is covalently bound to an albumin -binding moiety
  MOD_RES 38: AMIDATION

SEQ ID NO: 51 - protein, 38 aa, synthetic construct; identical to SEQ ID NO: 11
  MOD_RES 1: ACETYLATION
  VARIANT 7: D-valine
  MOD_RES 12: the epsilon-amino group of the lysine side chain is covalently bound to an albumin -binding moiety
  VARIANT 32: X is Abu
  MOD_RES 38: AMIDATION

SEQ ID NO: 52 - protein, 38 aa, synthetic construct; identical to SEQ ID NO: 11
  MOD_RES 1: ACETYLATION
  VARIANT 7: D-valine
  MOD_RES 12: the epsilon-amino group of the lysine side chain is covalently bound to an albumin -binding moiety
  VARIANT 32: X is Nva
  MOD_RES 38: AMIDATION

SEQ ID NO: 53 - protein, 38 aa, synthetic construct
  MOD_RES 1: ACETYLATION
  VARIANT 7: D-valine
  VARIANT 11: X is alpha-methyl-leucine
  MOD_RES 12: the epsilon-amino group of the lysine side chain is covalently bound to an albumin -binding moiety
  MOD_RES 38: AMIDATION
IVLSLDVPIKXKKILLEQEKQKKQREQAETDKQILAQV

SEQ ID NO: 54 - protein, 39 aa, synthetic construct
  MOD_RES 1: ACETYLATION
  VARIANT 7: D-valine
  MOD_RES 12: the epsilon-amino group of the lysine side chain is covalently bound to an albumin -binding moiety
  VARIANT 32: X is alpha-methyl-leucine
  MOD_RES 38: AMIDATION
IVLSLDVPIKLKKILLEQEKQKKQREQAETNXKQILAQV

SEQ ID NO: 55 - protein, 38 aa, synthetic construct; identical to SEQ ID NO: 11
  MOD_RES 1: ACETYLATION
  VARIANT 7: D-valine
  MOD_RES 12: the epsilon-amino group of the lysine side chain is covalently bound to an albumin -binding moiety
  VARIANT 32: X is Dap
  MOD_RES 38: AMIDATION

SEQ ID NO: 56 - protein, 38 aa, synthetic construct
  MOD_RES 1: ACETYLATION
  VARIANT 7: D-valine
  MOD_RES 12: the epsilon-amino group of the lysine side chain is covalently bound to an albumin -binding moiety
  MOD_RES 38: AMIDATION
IVLSLDVPIKLKKILLEQEKQKKQREQAETNEQILAQV

SEQ ID NO: 57 - protein, 38 aa, synthetic construct; identical to SEQ ID NO: 11
  MOD_RES 1: ACETYLATION
  VARIANT 7: D-valine
  MOD_RES 12: the epsilon-amino group of the lysine side chain is covalently bound to an albumin -binding moiety
  VARIANT 32: X is 4-Pip
  MOD_RES 38: AMIDATION

SEQ ID NO: 58 - protein, 38 aa, synthetic construct; identical to SEQ ID NO: 11
  MOD_RES 1: ACETYLATION
  VARIANT 7: D-valine
  MOD_RES 12: the epsilon-amino group of the lysine side chain is covalently bound to an albumin -binding moiety
  VARIANT 32: X is Thp
  MOD_RES 38: AMIDATION

SEQ ID NO: 59 - protein, 38 aa, synthetic construct; identical to SEQ ID NO: 11
  MOD_RES 1: ACETYLATION
  VARIANT 7: D-valine
  MOD_RES 12: the epsilon-amino group of the lysine side chain is covalently bound to an albumin -binding moiety
  VARIANT 32: X is Chx
  MOD_RES 38: AMIDATION

SEQ ID NO: 60 - protein, 38 aa, synthetic construct; identical to SEQ ID NO: 11
  MOD_RES 1: ACETYLATION
  VARIANT 7: D-valine
  MOD_RES 12: the epsilon-amino group of the lysine side chain is covalently bound to an albumin -binding moiety
  VARIANT 32: X is Cpex
  MOD_RES 38: AMIDATION

SEQ ID NO: 61 - protein, 38 aa, synthetic construct; identical to SEQ ID NO: 11
  MOD_RES 1: ACETYLATION
  VARIANT 7: D-valine
  MOD_RES 12: the epsilon-amino group of the lysine side chain is covalently bound to an albumin -binding moiety
  VARIANT 32: X is Cpx
  MOD_RES 38: AMIDATION

SEQ ID NO: 62 - protein, 38 aa, synthetic construct
  MOD_RES 1: ACETYLATION
  VARIANT 7: D-valine
  MOD_RES 12: the epsilon-amino group of the lysine side chain is covalently bound to an albumin -binding moiety
  VARIANT 32: X is 4-Pip
  MOD_RES 38: AMIDATION
IVLSLDVPIKLKKILLEQEKQKAQREQAETNXQILAQV

SEQ ID NO: 63 - protein, 38 aa, synthetic construct
  MOD_RES 1: ACETYLATION
  VARIANT 7: D-valine
  MOD_RES 12: the epsilon-amino group of the lysine side chain is covalently bound to an albumin -binding moiety
  VARIANT 23: X is Aib
  VARIANT 32: X is 4-Pip
IVLSLDVPIKLKKILLEQEKQKXQREQAETNXQILAQV

SEQ ID NO: 64 - protein, 38 aa, synthetic construct; identical to SEQ ID NO: 11
  MOD_RES 1: METHYLATION
  VARIANT 7: D-valine
  MOD_RES 12: the epsilon-amino group of the lysine side chain is covalently bound to an albumin -binding moiety
  VARIANT 32: X is Aib
  MOD_RES 38: AMIDATION

SEQ ID NO: 65 - protein, 38 aa, synthetic construct; identical to SEQ ID NO: 38
  MOD_RES 1: METHYLATION
  VARIANT 7: D-valine
  VARIANT 11: X is alpha-methyl-leucine
  MOD_RES 12: the epsilon-amino group of the lysine side chain is covalently bound to an albumin -binding moiety
  VARIANT 32: X is Aib
  MOD_RES 38: AMIDATION

SEQ ID NO: 66 - protein, 38 aa, synthetic construct; identical to SEQ ID NO: 48
  MOD_RES 1: METHYLATION
  VARIANT 7: D-valine
  MOD_RES 12: the epsilon-amino group of the lysine side chain is covalently bound to an albumin -binding moiety
  MOD_RES 38: AMIDATION

SEQ ID NO: 67 - protein, 38 aa, synthetic construct; identical to SEQ ID NO: 49
  MOD_RES 1: METHYLATION
  VARIANT 7: D-valine
  VARIANT 11: X is alpha-methyl-leucine
  MOD_RES 12: the epsilon-amino group of the lysine side chain is covalently bound to an albumin -binding moiety
  MOD_RES 38: AMIDATION

SEQ ID NO: 68 - protein, 38 aa, synthetic construct; identical to SEQ ID NO: 47
  MOD_RES 1: METHYLATION
  VARIANT 7: D-valine
  MOD_RES 12: the epsilon-amino group of the lysine side chain is covalently bound to an albumin -binding moiety
  MOD_RES 38: AMIDATION

SEQ ID NO: 69 - protein, 38 aa, synthetic construct; identical to SEQ ID NO: 11
  MOD_RES 1: METHYLATION
  VARIANT 7: D-valine
  MOD_RES 12: the epsilon-amino group of the lysine side chain is covalently bound to an albumin -binding moiety
  VARIANT 32: X is Abu
  MOD_RES 38: AMIDATION

SEQ ID NO: 70 - protein, 38 aa, synthetic construct; identical to SEQ ID NO: 11
  MOD_RES 1: METHYLATION
  VARIANT 7: D-valine
  MOD_RES 12: the epsilon-amino group of the lysine side chain is covalently bound to an albumin -binding moiety
  VARIANT 32: X is Dap
  MOD_RES 38: AMIDATION

SEQ ID NO: 71 - protein, 38 aa, synthetic construct; identical to SEQ ID NO: 56
  MOD_RES 1: METHYLATION
  VARIANT 7: D-valine
  MOD_RES 12: the epsilon-amino group of the lysine side chain is covalently bound to an albumin -binding moiety
  MOD_RES 38: AMIDATION

SEQ ID NO: 72 - protein, 38 aa, synthetic construct; identical to SEQ ID NO: 11
  MOD_RES 1: METHYLATION
  VARIANT 7: D-valine
  MOD_RES 12: the epsilon-amino group of the lysine side chain is covalently bound to an albumin -binding moiety
  VARIANT 32: X is 4-Pip
  MOD_RES 38: AMIDATION

SEQ ID NO: 73 - protein, 38 aa, synthetic construct; identical to SEQ ID NO: 11
  MOD_RES 1: METHYLATION
  VARIANT 7: D-valine
  MOD_RES 12: the epsilon-amino group of the lysine side chain is covalently bound to an albumin -binding moiety
  VARIANT 32: X is Thp
  MOD_RES 38: AMIDATION

SEQ ID NO: 74 - protein, 38 aa, synthetic construct; identical to SEQ ID NO: 62
  MOD_RES 1: METHYLATION
  VARIANT 7: D-valine
  MOD_RES 12: the epsilon-amino group of the lysine side chain is covalently bound to an albumin -binding moiety
  VARIANT 32: X is Aib
  MOD_RES 38: AMIDATION

SEQ ID NO: 75 - protein, 38 aa, synthetic construct; identical to SEQ ID NO: 63
  MOD_RES 1: METHYLATION
  VARIANT 7: D-valine
  MOD_RES 12: the epsilon-amino group of the lysine side chain is covalently bound to an albumin -binding moiety
  VARIANT 23: X is Aib
  VARIANT 32: X is Aib

SEQ ID NO: 76 - protein, 38 aa, synthetic construct; identical to SEQ ID NO: 62
  MOD_RES 1: METHYLATION
  VARIANT 7: D-valine
  MOD_RES 12: the epsilon-amino group of the lysine side chain is covalently bound to an albumin -binding moiety
  VARIANT 32: X is 4-Pip
  MOD_RES 38: AMIDATION

SEQ ID NO: 77 - protein, 38 aa, synthetic construct; identical to SEQ ID NO: 63
  MOD_RES 1: METHYLATION
  VARIANT 7: D-valine
  MOD_RES 12: the epsilon-amino group of the lysine side chain is covalently bound to an albumin -binding moiety
  VARIANT 23: X is Aib
  VARIANT 32: X is 4-Pip

SEQ ID NO: 78 - protein, 37 aa, synthetic construct; identical to SEQ ID NO: 45
  MOD_RES 1: Acetylated with a propanoyl group
  VARIANT 6: D-valine
  MOD_RES 11: the epsilon-amino group of the lysine side chain is covalently bound to an albumin -binding moiety
  VARIANT 31: X is Aib
  MOD_RES 37: AMIDATION

SEQ ID NO: 79 - protein, 37 aa, synthetic construct; identical to SEQ ID NO: 45
  MOD_RES 1: Acetylated with a butanoyl group
  VARIANT 6: D-valine
  MOD_RES 11: the epsilon-amino group of the lysine side chain is covalently bound to an albumin -binding moiety
  VARIANT 31: X is Aib
  MOD_RES 37: AMIDATION

SEQ ID NO: 80 - protein, 37 aa, synthetic construct; identical to SEQ ID NO: 45
  MOD_RES 1: Acetylated with a pentanoyl group
  VARIANT 6: D-valine
  MOD_RES 11: the epsilon-amino group of the lysine side chain is covalently bound to an albumin -binding moiety
  VARIANT 31: X is Aib
  MOD_RES 37: AMIDATION

SEQ ID NO: 81 - protein, 37 aa, synthetic construct
  MOD_RES 1: Acetylated with a pentanoyl group
  VARIANT 6: D-valine
  MOD_RES 11: the epsilon-amino group of the lysine side chain is covalently bound to an albumin -binding moiety
  MOD_RES 37: AMIDATION
VLSLDVPIKLKKILLEQEKQKKQREQAETNVQILAQV

SEQ ID NO: 82 - protein, 38 aa, synthetic construct; identical to SEQ ID NO: 11
  MOD_RES 1: ACETYLATION
  VARIANT 7: D-valine
  MOD_RES 12: the epsilon-amino group of the lysine side chain is covalently bound to an albumin -binding moiety
  VARIANT 32: X is Aib
  MOD_RES 38: AMIDATION

SEQ ID NO: 83 - protein, 38 aa, synthetic construct; identical to SEQ ID NO: 11
  MOD_RES 1: ACETYLATION
  VARIANT 7: D-valine
  MOD_RES 12: the epsilon-amino group of the lysine side chain is covalently bound to an albumin -binding moiety
  VARIANT 32: X is Abu
  MOD_RES 38: AMIDATION

SEQ ID NO: 84 - protein, 38 aa, synthetic construct; identical to SEQ ID NO: 11
  MOD_RES 1: ACETYLATION
  VARIANT 7: D-valine
  MOD_RES 12: the epsilon-amino group of the lysine side chain is covalently bound to an albumin -binding moiety
  VARIANT 32: X is 4-Pip
  MOD_RES 38: AMIDATION

SEQ ID NO: 85 - protein, 38 aa, synthetic construct; identical to SEQ ID NO: 56
  MOD_RES 1: ACETYLATION
  VARIANT 7: D-valine
  MOD_RES 12: the epsilon-amino group of the lysine side chain is covalently bound to an albumin -binding moiety
  MOD_RES 38: AMIDATION

SEQ ID NO: 86 - protein, 37 aa, synthetic construct; identical to SEQ ID NO: 45
  MOD_RES 1: Acetylated with a pentanoyl group
  VARIANT 6: D-valine
  MOD_RES 11: the epsilon-amino group of the lysine side chain is covalently bound to an albumin -binding moiety
  VARIANT 31: X is Aib
  MOD_RES 37: AMIDATION

SEQ ID NO: 87 - protein, 38 aa, synthetic construct; identical to SEQ ID NO: 11
  MOD_RES 1: METHYLATION
  VARIANT 7: D-valine
  MOD_RES 12: the epsilon-amino group of the lysine side chain is covalently bound to an albumin -binding moiety
  VARIANT 32: X is Aib
  MOD_RES 38: AMIDATION

SEQ ID NO: 88 - protein, 38 aa, synthetic construct; identical to SEQ ID NO: 62
  MOD_RES 1: METHYLATION
  VARIANT 7: D-valine
  MOD_RES 12: the epsilon-amino group of the lysine side chain is covalently bound to an albumin -binding moiety
  VARIANT 32: X is Aib
  MOD_RES 38: AMIDATION

SEQ ID NO: 89 - protein, 38 aa, synthetic construct; identical to SEQ ID NO: 63
  MOD_RES 1: METHYLATION
  VARIANT 7: D-valine
  MOD_RES 12: the epsilon-amino group of the lysine side chain is covalently bound to an albumin -binding moiety
  VARIANT 23: X is Aib
  VARIANT 32: X is Aib
  MOD_RES 38: AMIDATION

SEQ ID NO: 90 - protein, 38 aa, synthetic construct; identical to SEQ ID NO: 62
  MOD_RES 1: ACETYLATION
  VARIANT 7: D-valine
  MOD_RES 12: the epsilon-amino group of the lysine side chain is covalently bound to an albumin -binding moiety
  VARIANT 32: X is 4-Pip
  MOD_RES 38: AMIDATION

SEQ ID NO: 91 - protein, 38 aa, synthetic construct; identical to SEQ ID NO: 63
  MOD_RES 1: ACETYLATION
  VARIANT 7: D-valine
  MOD_RES 12: the epsilon-amino group of the lysine side chain is covalently bound to an albumin -binding moiety
  VARIANT 23: X is Aib
  VARIANT 32: X is 4-Pip
  MOD_RES 38: AMIDATION

SEQ ID NO: 92 - protein, 37 aa, synthetic construct; identical to SEQ ID NO: 33
  MOD_RES 1: ACETYLATION
  VARIANT 6: D-valine
  MOD_RES 11: the epsilon-amino group of the lysine side chain is covalently bound to an albumin -binding moiety
  MOD_RES 37: AMIDATION

SEQ ID NO: 93 - protein, 37 aa, synthetic construct; identical to SEQ ID NO: 33
  VARIANT 6: D-valine
  MOD_RES 11: the epsilon-amino group of the lysine side chain is covalently bound to an albumin -binding moiety
  MOD_RES 37: AMIDATION

SEQ ID NO: 94 - protein, 37 aa, synthetic construct; identical to SEQ ID NO: 33
  MOD_RES 1: Acetylated with a propanoyl group
  MOD_RES 11: the epsilon-amino group of the lysine side chain is covalently bound to an albumin -binding moiety
  MOD_RES 37: AMIDATION

SEQ ID NO: 95 - protein, 37 aa, synthetic construct; identical to SEQ ID NO: 33
  MOD_RES 1: Acetylated with a butanoyl group
  MOD_RES 11: the epsilon-amino group of the lysine side chain is covalently bound to an albumin -binding moiety
  MOD_RES 37: AMIDATION

SEQ ID NO: 96 - protein, 37 aa, synthetic construct; identical to SEQ ID NO: 33
  MOD_RES 1: Acetylated with a pentanoyl group
  MOD_RES 11: the epsilon-amino group of the lysine side chain is covalently bound to an albumin -binding moiety
  MOD_RES 37: AMIDATION

SEQ ID NO: 97 - protein, 38 aa, synthetic construct; identical to SEQ ID NO: 11
  MOD_RES 1: ACETYLATION
  MOD_RES 12: the epsilon-amino group of the lysine side chain is covalently bound to an albumin -binding moiety
  VARIANT 32: X is Aib
  MOD_RES 38: AMIDATION

SEQ ID NO: 98 - protein, 38 aa, synthetic construct; identical to SEQ ID NO: 11
  MOD_RES 1: ACETYLATION
  VARIANT 7: D-valine
  MOD_RES 12: the epsilon-amino group of the lysine side chain is covalently bound to an albumin -binding moiety
  VARIANT 32: X is Aib
  MOD_RES 38: AMIDATION

SEQ ID NO: 99 - protein, 37 aa, synthetic construct; identical to SEQ ID NO: 45
  MOD_RES 1: ACETYLATION
  VARIANT 6: D-valine
  MOD_RES 11: the epsilon-amino group of the lysine side chain is covalently bound to an albumin -binding moiety
  VARIANT 31: X is Aib
  MOD_RES 37: AMIDATION

SEQ ID NO: 100 - protein, 38 aa, synthetic construct; identical to SEQ ID NO: 47
  MOD_RES 1: ACETYLATION
  VARIANT 7: D-valine
  MOD_RES 12: the epsilon-amino group of the lysine side chain is covalently bound to an albumin -binding moiety
  MOD_RES 38: AMIDATION

SEQ ID NO: 101 - protein, 37 aa, synthetic construct
  MOD_RES 1: ACETYLATION
  VARIANT 6: D-valine
  MOD_RES 11: the epsilon-amino group of the lysine side chain is covalently bound to an albumin -binding moiety
  MOD_RES 37: AMIDATION
VLSLDVPIKLKKILLEQEKQKKQREQAETNAQILAQV

SEQ ID NO: 102 - protein, 38 aa, synthetic construct; identical to SEQ ID NO: 48
  MOD_RES 1: ACETYLATION
  MOD_RES 12: the epsilon-amino group of the lysine side chain is covalently bound to an albumin -binding moiety
  MOD_RES 38: AMIDATION

SEQ ID NO: 103 - protein, 38 aa, synthetic construct; identical to SEQ ID NO: 48
  MOD_RES 1: ACETYLATION
  VARIANT 7: D-valine
  MOD_RES 12: the epsilon-amino group of the lysine side chain is covalently bound to an albumin -binding moiety
  MOD_RES 38: AMIDATION

SEQ ID NO: 104 - protein, 38 aa, synthetic construct; identical to SEQ ID NO: 11
  MOD_RES 1: ACETYLATION
  VARIANT 7: D-valine
  MOD_RES 12: the epsilon-amino group of the lysine side chain is covalently bound to an albumin -binding moiety
  VARIANT 32: X is Abu
  MOD_RES 38: AMIDATION

SEQ ID NO: 105 - protein, 38 aa, synthetic construct; identical to SEQ ID NO: 11
  MOD_RES 1: ACETYLATION
  VARIANT 7: D-valine
  MOD_RES 12: the epsilon-amino group of the lysine side chain is covalently bound to an albumin -binding moiety
  VARIANT 32: X is Nva
  MOD_RES 38: AMIDATION

SEQ ID NO: 106 - protein, 38 aa, synthetic construct; identical to SEQ ID NO: 11
  MOD_RES 1: ACETYLATION
  VARIANT 7: D-valine
  MOD_RES 12: the epsilon-amino group of the lysine side chain is covalently bound to an albumin -binding moiety
  VARIANT 31: X is alpha-methyl-leucine
  MOD_RES 38: AMIDATION

SEQ ID NO: 107 - protein, 38 aa, synthetic construct; identical to SEQ ID NO: 11
  MOD_RES 1: ACETYLATION
  VARIANT 7: D-valine
  MOD_RES 12: the epsilon-amino group of the lysine side chain is covalently bound to an albumin -binding moiety
  VARIANT 32: X is Dap
  MOD_RES 38: AMIDATION

SEQ ID NO: 108 - protein, 38 aa, synthetic construct; identical to SEQ ID NO: 56
  MOD_RES 1: ACETYLATION
  VARIANT 7: D-valine
  MOD_RES 12: the epsilon-amino group of the lysine side chain is covalently bound to an albumin -binding moiety
  MOD_RES 38: AMIDATION

SEQ ID NO: 109 - protein, 38 aa, synthetic construct; identical to SEQ ID NO: 11
  MOD_RES 1: ACETYLATION
  VARIANT 7: D-valine
  MOD_RES 12: the epsilon-amino group of the lysine side chain is covalently bound to an albumin -binding moiety
  VARIANT 32: X is 4-Pip
  MOD_RES 38: AMIDATION

SEQ ID NO: 110 - protein, 38 aa, synthetic construct; identical to SEQ ID NO: 38
  MOD_RES 1: ACETYLATION
  VARIANT 7: D-valine
  VARIANT 11: X is alpha-methyl-leucine
  MOD_RES 12: the epsilon-amino group of the lysine side chain is covalently bound to an albumin -binding moiety
  VARIANT 32: X is Aib
  MOD_RES 38: AMIDATION

SEQ ID NO: 111 - protein, 38 aa, synthetic construct; identical to SEQ ID NO: 49
  MOD_RES 1: ACETYLATION
  VARIANT 7: D-valine
  VARIANT 11: X is alpha-methyl-leucine
  MOD_RES 12: the epsilon-amino group of the lysine side chain is covalently bound to an albumin -binding moiety
  MOD_RES 38: AMIDATION

SEQ ID NO: 112 - protein, 38 aa, synthetic construct
  MOD_RES 1: ACETYLATION
  VARIANT 7: D-valine
  VARIANT 11: X is alpha-methyl-leucine
  MOD_RES 12: the epsilon-amino group of the lysine side chain is covalently bound to an albumin -binding moiety
  MOD_RES 38: AMIDATION
IVLSLDVPIKXKKILLEQEKQKKQREQAETNAQILAQV

SEQ ID NO: 113 - protein, 38 aa, synthetic construct; identical to SEQ ID NO: 47
  MOD_RES 1: METHYLATION
  VARIANT 7: D-valine
  MOD_RES 12: the epsilon-amino group of the lysine side chain is covalently bound to an albumin -binding moiety
  MOD_RES 38: AMIDATION

SEQ ID NO: 114 - protein, 38 aa, synthetic construct; identical to SEQ ID NO: 11
  MOD_RES 1: METHYLATION
  VARIANT 7: D-valine
  MOD_RES 12: the epsilon-amino group of the lysine side chain is covalently bound to an albumin -binding moiety
  VARIANT 32: X is Abu
  MOD_RES 38: AMIDATION

SEQ ID NO: 115 - protein, 38 aa, synthetic construct; identical to SEQ ID NO: 11
  MOD_RES 1: METHYLATION
  VARIANT 7: D-valine
  MOD_RES 12: the epsilon-amino group of the lysine side chain is covalently bound to an albumin -binding moiety
  VARIANT 32: X is Dap
  MOD_RES 38: AMIDATION

SEQ ID NO: 116 - protein, 38 aa, synthetic construct; identical to SEQ ID NO: 56
  MOD_RES 1: METHYLATION
  VARIANT 7: D-valine
  MOD_RES 12: the epsilon-amino group of the lysine side chain is covalently bound to an albumin -binding moiety
  MOD_RES 38: AMIDATION

SEQ ID NO: 117 - protein, 38 aa, synthetic construct; identical to SEQ ID NO: 11
  MOD_RES 1: METHYLATION
  VARIANT 7: D-valine
  MOD_RES 12: the epsilon-amino group of the lysine side chain is covalently bound to an albumin -binding moiety
  VARIANT 32: X is 4-Pip
  MOD_RES 38: AMIDATION

SEQ ID NO: 118 - protein, 38 aa, synthetic construct; identical to SEQ ID NO: 11
  MOD_RES 1: METHYLATION
  VARIANT 7: D-valine
  MOD_RES 12: the epsilon-amino group of the lysine side chain is covalently bound to an albumin -binding moiety
  VARIANT 32: X is Aib
  MOD_RES 38: AMIDATION

SEQ ID NO: 119 - protein, 38 aa, synthetic construct; identical to SEQ ID NO: 38
  MOD_RES 1: METHYLATION
  VARIANT 7: D-valine
  VARIANT 11: X is alpha-methyl-leucine
  MOD_RES 12: the epsilon-amino group of the lysine side chain is covalently bound to an albumin -binding moiety
  VARIANT 32: X is Aib
  MOD_RES 38: AMIDATION

SEQ ID NO: 120 - protein, 37 aa, synthetic construct; identical to SEQ ID NO: 45
  MOD_RES 1: Acetylated with a pentanoyl group
  VARIANT 6: D-valine
  MOD_RES 11: the epsilon-amino group of the lysine side chain is covalently bound to an albumin -binding moiety
  VARIANT 31: X is Aib
  MOD_RES 37: AMIDATION

SEQ ID NO: 121 - protein, 37 aa, synthetic construct; identical to SEQ ID NO: 81
  MOD_RES 1: Acetylated with a pentanoyl group
  VARIANT 6: D-valine
  MOD_RES 11: the epsilon-amino group of the lysine side chain is covalently bound to an albumin -binding moiety
  MOD_RES 37: AMIDATION

SEQ ID NO: 122 - protein, 37 aa, synthetic construct; identical to SEQ ID NO: 101
  MOD_RES 1: Acetylated with a pentanoyl group
  VARIANT 6: D-valine
  MOD_RES 11: the epsilon-amino group of the lysine side chain is covalently bound to an albumin -binding moiety
  MOD_RES 37: AMIDATION

SEQ ID NO: 123 - protein, 37 aa, synthetic construct; identical to SEQ ID NO: 46
  MOD_RES 1: Acetylated with a pentanoyl group
  VARIANT 6: D-valine
  MOD_RES 11: the epsilon-amino group of the lysine side chain is covalently bound to an albumin -binding moiety
  VARIANT 11: X is alpha-methyl-leucine
  VARIANT 31: X is Aib
  MOD_RES 37: AMIDATION

SEQ ID NO: 124 - protein, 37 aa, synthetic construct
  MOD_RES 1: Acetylated with a pentanoyl group
  VARIANT 7: D-valine
  VARIANT 10: X is alpha-methyl-leucine
  MOD_RES 11: the epsilon-amino group of the lysine side chain is covalently bound to an albumin -binding moiety
  MOD_RES 37: AMIDATION
VLSLDVPIKXKKILLEQEKQKKQREQAETNVQILAQV

SEQ ID NO: 125 - protein, 38 aa, synthetic construct; identical to SEQ ID NO: 11
  MOD_RES 1: ACETYLATION
  VARIANT 7: D-valine
  MOD_RES 12: the epsilon-amino group of the lysine side chain is covalently bound to an albumin -binding moiety
  VARIANT 32: X is Aib
  MOD_RES 38: AMIDATION

SEQ ID NO: 126 - protein, 38 aa, synthetic construct; identical to SEQ ID NO: 47
  MOD_RES 1: ACETYLATION
  VARIANT 7: D-valine
  MOD_RES 12: the epsilon-amino group of the lysine side chain is covalently bound to an albumin -binding moiety
  MOD_RES 38: AMIDATION

SEQ ID NO: 127 - protein, 38 aa, synthetic construct; identical to SEQ ID NO: 11
  MOD_RES 1: ACETYLATION
  VARIANT 7: D-valine
  MOD_RES 12: the epsilon-amino group of the lysine side chain is covalently bound to an albumin -binding moiety
  VARIANT 32: X is Abu
  MOD_RES 38: AMIDATION

SEQ ID NO: 128 - protein, 38 aa, synthetic construct; identical to SEQ ID NO: 11
  MOD_RES 1: ACETYLATION
  VARIANT 7: D-valine
  MOD_RES 12: the epsilon-amino group of the lysine side chain is covalently bound to an albumin -binding moiety
  VARIANT 32: X is Dap
  MOD_RES 38: AMIDATION

SEQ ID NO: 129 - protein, 38 aa, synthetic construct; identical to SEQ ID NO: 11
  MOD_RES 1: ACETYLATION
  VARIANT 7: D-valine
  MOD_RES 12: the epsilon-amino group of the lysine side chain is covalently bound to an albumin -binding moiety
  VARIANT 32: X is 4-Pip
  MOD_RES 38: AMIDATION

SEQ ID NO: 130 - protein, 38 aa, synthetic construct; identical to SEQ ID NO: 56
  MOD_RES 1: ACETYLATION
  VARIANT 7: D-valine
  MOD_RES 12: the epsilon-amino group of the lysine side chain is covalently bound to an albumin -binding moiety
  MOD_RES 38: AMIDATION

SEQ ID NO: 131 - protein, 38 aa, synthetic construct; identical to SEQ ID NO: 62
  MOD_RES 1: ACETYLATION
  VARIANT 7: D-valine
  MOD_RES 12: the epsilon-amino group of the lysine side chain is covalently bound to an albumin -binding moiety
  VARIANT 32: X is 4-Pip
  MOD_RES 38: AMIDATION

SEQ ID NO: 132 - protein, 38 aa, synthetic construct; identical to SEQ ID NO: 63
  MOD_RES 1: ACETYLATION
  VARIANT 7: D-valine
  MOD_RES 12: the epsilon-amino group of the lysine side chain is covalently bound to an albumin -binding moiety
  VARIANT 23: X is Aib
  VARIANT 32: X is 4-Pip
  MOD_RES 38: AMIDATION

SEQ ID NO: 133 - protein, 38 aa, synthetic construct; identical to SEQ ID NO: 11
  MOD_RES 1: ACETYLATION
  VARIANT 7: D-valine
  MOD_RES 12: the epsilon-amino group of the lysine side chain is covalently bound to an albumin -binding moiety
  VARIANT 32: X is Thp
  MOD_RES 38: AMIDATION

SEQ ID NO: 134 - protein, 38 aa, synthetic construct; identical to SEQ ID NO: 11
  MOD_RES 1: ACETYLATION
  VARIANT 7: D-valine
  MOD_RES 12: the epsilon-amino group of the lysine side chain is covalently bound to an albumin -binding moiety
  VARIANT 32: X is Chx
  MOD_RES 38: AMIDATION

SEQ ID NO: 135 - protein, 38 aa, synthetic construct; identical to SEQ ID NO: 11
  MOD_RES 1: ACETYLATION
  VARIANT 7: D-valine
  MOD_RES 12: the epsilon-amino group of the lysine side chain is covalently bound to an albumin -binding moiety
  VARIANT 32: X is Cpex
  MOD_RES 38: AMIDATION

SEQ ID NO: 136 - protein, 38 aa, synthetic construct; identical to SEQ ID NO: 11
  MOD_RES 1: ACETYLATION
  VARIANT 7: D-valine
  MOD_RES 12: the epsilon-amino group of the lysine side chain is covalently bound to an albumin -binding moiety
  VARIANT 32: X is Cpx
  MOD_RES 38: AMIDATION

SEQ ID NO: 137 - protein, 38 aa, synthetic construct; identical to SEQ ID NO: 11
  MOD_RES 1: METHYLATION
  VARIANT 7: D-valine
  MOD_RES 12: the epsilon-amino group of the lysine side chain is covalently bound to an albumin -binding moiety
  VARIANT 32: X is Aib
  MOD_RES 38: AMIDATION

SEQ ID NO: 138 - protein, 38 aa, synthetic construct; identical to SEQ ID NO: 47
  MOD_RES 1: METHYLATION
  VARIANT 7: D-valine
  MOD_RES 12: the epsilon-amino group of the lysine side chain is covalently bound to an albumin -binding moiety
  MOD_RES 38: AMIDATION

SEQ ID NO: 139 - protein, 38 aa, synthetic construct; identical to SEQ ID NO: 11
  MOD_RES 1: METHYLATION
  VARIANT 7: D-valine
  MOD_RES 12: the epsilon-amino group of the lysine side chain is covalently bound to an albumin -binding moiety
  VARIANT 32: X is Abu
  MOD_RES 38: AMIDATION

SEQ ID NO: 140 - protein, 38 aa, synthetic construct; identical to SEQ ID NO: 11
  MOD_RES 1: METHYLATION
  VARIANT 7: D-valine
  MOD_RES 12: the epsilon-amino group of the lysine side chain is covalently bound to an albumin -binding moiety
  VARIANT 32: X is Dap
  MOD_RES 38: AMIDATION

SEQ ID NO: 141 - protein, 38 aa, synthetic construct; identical to SEQ ID NO: 11
  MOD_RES 1: METHYLATION
  VARIANT 7: D-valine
  MOD_RES 12: the epsilon-amino group of the lysine side chain is covalently bound to an albumin -binding moiety
  VARIANT 32: X is 4-Pip
  MOD_RES 38: AMIDATION

SEQ ID NO: 142 - protein, 38 aa, synthetic construct; identical to SEQ ID NO: 56
  MOD_RES 1: METHYLATION
  VARIANT 7: D-valine
  MOD_RES 12: the epsilon-amino group of the lysine side chain is covalently bound to an albumin -binding moiety
  MOD_RES 38: AMIDATION

SEQ ID NO: 143 - protein, 38 aa, synthetic construct; identical to SEQ ID NO: 11
  MOD_RES 1: METHYLATION
  VARIANT 7: D-valine
  MOD_RES 12: the epsilon-amino group of the lysine side chain is covalently bound to an albumin -binding moiety
  VARIANT 32: X is Thp
  MOD_RES 38: AMIDATION

SEQ ID NO: 144 - protein, 38 aa, synthetic construct; identical to SEQ ID NO: 62
  MOD_RES 1: METHYLATION
  VARIANT 7: D-valine
  MOD_RES 12: the epsilon-amino group of the lysine side chain is covalently bound to an albumin -binding moiety
  VARIANT 32: X is Aib
  MOD_RES 38: AMIDATION

SEQ ID NO: 145 - protein, 38 aa, synthetic construct; identical to SEQ ID NO: 63
  MOD_RES 1: METHYLATION
  VARIANT 7: D-valine
  MOD_RES 12: the epsilon-amino group of the lysine side chain is covalently bound to an albumin -binding moiety
  VARIANT 23: X is Aib
  VARIANT 32: X is Aib
  MOD_RES 38: AMIDATION

SEQ ID NO: 146 - protein, 38 aa, synthetic construct
  Comp 3
  VARIANT 7: D-valine
  MOD_RES 12: the epsilon-amino group of the lysine side chain is covalently bound to an albumin -binding moiety
  MOD_RES 38: AMIDATION
IVLSLDVPIKLKQILLKQERQKKQREQAEKNKQILEQV

SEQ ID NO: 147 - protein, 38 aa, synthetic construct; identical to SEQ ID NO: 146
  Comp 2
  VARIANT 7: D-valine
  MOD_RES 12: the epsilon-amino group of the lysine side chain is covalently bound to an albumin -binding moiety
  MOD_RES 38: AMIDATION

SEQ ID NO: 148 - protein, 38 aa, synthetic construct; identical to SEQ ID NO: 146
  VARIANT 7: D-valine
  MOD_RES 12: the epsilon-amino group of the lysine side chain is covalently bound to an albumin -binding moiety
  MOD_RES 38: AMIDATION

SEQ ID NO: 149 - protein, 38 aa, synthetic construct
  VARIANT 7: D-valine
  MOD_RES 12: the epsilon-amino group of the lysine side chain is covalently bound to an albumin -binding moiety
  MOD_RES 38: AMIDATION
IVLSLDVPIKLKKILLEQEKQKKQREQAETNKQILAQV

SEQ ID NO: 150 - protein, 38 aa, synthetic construct; identical to SEQ ID NO: 146
  VARIANT 7: D-valine
  MOD_RES 12: the epsilon-amino group of the lysine side chain is covalently bound to an albumin -binding moiety
  MOD_RES 38: AMIDATION

SEQ ID NO: 151 - protein, 38 aa, synthetic construct; identical to SEQ ID NO: 146
  VARIANT 7: D-valine
  MOD_RES 12: the epsilon-amino group of the lysine side chain is covalently bound to an albumin -binding moiety
  MOD_RES 38: AMIDATION